European Patent Application EP 4 806 514 A2, published September 16, 2026. Title: ANTI-CDH17 ANTIBODIES AND USES THEREOF. Applicant: Concept to Medicine Biotech Co., Ltd. Application WO. The sequence listing filed with the application follows.

SEQUENCE LISTING (250 sequences)

SEQ ID NO: 1 - protein, 5 aa, synthetic construct
NYWMN

SEQ ID NO: 2 - protein, 17 aa, synthetic construct
TFNPSYGYTEYNQKFKD

SEQ ID NO: 3 - protein, 7 aa, synthetic construct
RSSHFDY

SEQ ID NO: 4 - protein, 17 aa, synthetic construct
KSSQSLLNSRTRTNYLA

SEQ ID NO: 5 - protein, 7 aa, synthetic construct
WASTRES

SEQ ID NO: 6 - protein, 8 aa, synthetic construct
KQSYNLPT

SEQ ID NO: 7 - protein, 116 aa, synthetic construct
QVQLQQSGAELAKPGTSVKMSCKASGYNFTNYWMNWVKQRPGQGLEWIGTFNPSYGYTEYNQKFKDKAILTADKSSSTAYMQLNSLTSEDSAVYYCARRSSHFDYWGQGTTLTVSS

SEQ ID NO: 8 - protein, 112 aa, synthetic construct
DIVMSQSPSSLAVSAGEKVTMSCKSSQSLLNSRTRTNYLAWYQQKPGQSPKLLIYWASTRESGVPDRFTGSGSGTDFTLTISSVQAEDLAVYYCKQSYNLPTFGGGTKLEIK

SEQ ID NO: 9 - protein, 5 aa, synthetic construct
SYGIS

SEQ ID NO: 10 - protein, 17 aa, synthetic construct
EIYPRSGNTYYNEKFKG

SEQ ID NO: 11 - protein, 10 aa, synthetic construct
LDYGTSPFDY

SEQ ID NO: 12 - protein, 11 aa, synthetic construct
KASENVGTFVS

SEQ ID NO: 13 - protein, 7 aa, synthetic construct
GASNRYT

SEQ ID NO: 14 - protein, 9 aa, synthetic construct
GQSYSYPYT

SEQ ID NO: 15 - protein, 119 aa, synthetic construct
QVQLQQSGAELARPGASVKLSCKASGYTFTSYGISWVKQRTGQGLEWIGEIYPRSGNTYYNEKFKGKATLTADKSSSTAYMELRSLTSEDSAVYFCSRLDYGTSPFDYWGQGTTLTVSS

SEQ ID NO: 16 - protein, 107 aa, synthetic construct
NIVMTQSPKSMSMSVGERVTLSCKASENVGTFVSWYQHKPEQSPKLLIYGASNRYTGVPDRFTGSGSATDFTLTISSVQAEDLADYHCGQSYSYPYTFGGGTKLEIK

SEQ ID NO: 17 - protein, 5 aa, synthetic construct
DYDMH

SEQ ID NO: 18 - protein, 17 aa, synthetic construct
GFDPESAGTVYNLRFKD

SEQ ID NO: 19 - protein, 12 aa, synthetic construct
KGYYSVSSPFTY

SEQ ID NO: 20 - protein, 17 aa, synthetic construct
KSSQSLLYSSNQKNYLA

SEQ ID NO: 21 - protein, 7 aa, synthetic construct
WASTRES

SEQ ID NO: 22 - protein, 9 aa, synthetic construct
QQCYSYPRT

SEQ ID NO: 23 - protein, 121 aa, synthetic construct
QVQLQQSGAELVRPGASVTLSCKASGYTFTDYDMHWVKQTPVHGLEWIGGFDPESAGTVYNLRFKDKAILTADKSSSTAYMELRSLTSEDSAVYYCARKGYYSVSSPFTYWGQGTLVSVSA

SEQ ID NO: 24 - protein, 113 aa, synthetic construct
DIGMSQSPSSLAVSVGEKVTMSCKSSQSLLYSSNQKNYLAWYQQKPGQSPKLLIYWASTRESGVPDRFTGSGSGTDFTLTINSVKAEDLAVYYCQQCYSYPRTFGGGTKLEIK

SEQ ID NO: 25 - protein, 5 aa, synthetic construct
DHTIH

SEQ ID NO: 26 - protein, 17 aa, synthetic construct
YIYPRDGYTKYNEKFKD

SEQ ID NO: 27 - protein, 10 aa, synthetic construct
FYYGYWYFDV

SEQ ID NO: 28 - protein, 16 aa, synthetic construct
RSSKSLLRSNGNTYLY

SEQ ID NO: 29 - protein, 7 aa, synthetic construct
RMSNLAS

SEQ ID NO: 30 - protein, 9 aa, synthetic construct
MQHLEYPFT

SEQ ID NO: 31 - protein, 119 aa, synthetic construct
QVQLQQSDAELVKPGASVKISCKVSGYTFTDHTIHWMKQRPEQGLEWIGYIYPRDGYTKYNEKFKDKATLTADKSSSTAYIQLNTLTSEDSAVYFCARFYYGYWYFDVWGTGTTVTVSS

SEQ ID NO: 32 - protein, 112 aa, synthetic construct
DIVMTQAAPSVPVTPGESVSISCRSSKSLLRSNGNTYLYWFLQRPGQSPQVLIYRMSNLASGVPDRFSGSGSGTAFTLRISRVEAEDVGVYYCMQHLEYPFTFGAGTKLELK

SEQ ID NO: 33 - protein, 5 aa, synthetic construct
SYAMS

SEQ ID NO: 34 - protein, 17 aa, synthetic construct
TINIGGSYTYYPDSVKG

SEQ ID NO: 35 - protein, 10 aa, synthetic construct
QEGRYWYFDV

SEQ ID NO: 36 - protein, 12 aa, synthetic construct
TASSSVSSSYLH

SEQ ID NO: 37 - protein, 7 aa, synthetic construct
STSNLAS

SEQ ID NO: 38 - protein, 9 aa, synthetic construct
HQFHRSPYT

SEQ ID NO: 39 - protein, 119 aa, synthetic construct
EVQLVESGGGLVKPGGSLKLSCAASGFTFSSYAMSWVRQTPEKRLEWVATINIGGSYTYYPDSVKGRFTISRDNAKNTLYLQMSSLRSEDTAMYYCARQEGRYWYFDVWGAGTTVTVSS

SEQ ID NO: 40 - protein, 108 aa, synthetic construct
QIVLTQSPAIMSASLGERVTMTCTASSSVSSSYLHWYQQKPGSSPKLWIYSTSNLASGVPARFSGSGSGTSYSLTISSMEAEDAATYYCHQFHRSPYTFGGGTKLEIK

SEQ ID NO: 41 - protein, 5 aa, synthetic construct
TYNMY

SEQ ID NO: 42 - protein, 17 aa, synthetic construct
YIDPYNGVTIYNQKFKG

SEQ ID NO: 43 - protein, 10 aa, synthetic construct
TAATLDAMDY

SEQ ID NO: 44 - protein, 11 aa, synthetic construct
KASQNVATAVA

SEQ ID NO: 45 - protein, 7 aa, synthetic construct
WTSTRHN

SEQ ID NO: 46 - protein, 9 aa, synthetic construct
QQYNSHPLT

SEQ ID NO: 47 - protein, 119 aa, synthetic construct
EIQLQQSGPELVKPGASVKVSCKASGYAFTTYNMYWVKQSHGQSLEWIGYIDPYNGVTIYNQKFKGTATLTVDKSSSTAYMHLNSLSSEDSAVYYCTITAATLDAMDYWGQGTSVTVSS

SEQ ID NO: 48 - protein, 107 aa, synthetic construct
DIVMTQSHKFMSTSVGDRVSITCKASQNVATAVAWYQQKPGQSPKVLIYWTSTRHNGVPDRFTGSGSGTDFTLTISNVQSEDLADYFCQQYNSHPLTFGAGTRLELK

SEQ ID NO: 49 - protein, 5 aa, synthetic construct
TYWMH

SEQ ID NO: 50 - protein, 17 aa, synthetic construct
EIDPSDSYANYNQKFKG

SEQ ID NO: 51 - protein, 6 aa, synthetic construct
YYGYGD

SEQ ID NO: 52 - protein, 12 aa, synthetic construct
SVSSSISSIHLH

SEQ ID NO: 53 - protein, 7 aa, synthetic construct
RTSNLAS

SEQ ID NO: 54 - protein, 9 aa, synthetic construct
QQGSNLPLT

SEQ ID NO: 55 - protein, 115 aa, synthetic construct
QVQLQQPGAELVKPGASVKLSCKASGYTFTTYWMHWVKQRPGQGLEWIGEIDPSDSYANYNQKFKGKATLTVDKSSSTAYMQLSSLTSEDSAVYYCALYYGYGDWGQGTTLTVSS

SEQ ID NO: 56 - protein, 108 aa, synthetic construct
EIVLTQSPTTMAASPGEKIIITCSVSSSISSIHLHWYQQKPGFSPKLLIYRTSNLASGVPTRFSGSGSGTSYSLTIGTMEAEDVATYYCQQGSNLPLTFGAGTRLELK

SEQ ID NO: 57 - protein, 5 aa, synthetic construct
GYWIE

SEQ ID NO: 58 - protein, 17 aa, synthetic construct
EILPGSGSTNYNEKFKG

SEQ ID NO: 59 - protein, 5 aa, synthetic construct
AGYNN

SEQ ID NO: 60 - protein, 11 aa, synthetic construct
RASQDIGRSVN

SEQ ID NO: 61 - protein, 7 aa, synthetic construct
ATSSLES

SEQ ID NO: 62 - protein, 9 aa, synthetic construct
LQYASSPLT

SEQ ID NO: 63 - protein, 114 aa, synthetic construct
QVQLQQSGAELMKPGASVKLSCKATGYTFTGYWIEWIKQRPGHGLEWIGEILPGSGSTNYNEKFKGKATFTADTSSNTAYMELSSLTTEDSAIYYCARAGYNNWGQGTTLTVSS

SEQ ID NO: 64 - protein, 107 aa, synthetic construct
DIQMTQSPSSLSASLGERVSLTCRASQDIGRSVNWLQQEPDGTIKRLIYATSSLESGVPKRFSGSRSGSDYFLTISSLESEDFVDYYCLQYASSPLTFGAGTKLELK

SEQ ID NO: 65 - protein, 5 aa, synthetic construct
DFYMA

SEQ ID NO: 66 - protein, 17 aa, synthetic construct
NINYDSTITYYLDSLKS

SEQ ID NO: 67 - protein, 12 aa, synthetic construct
LLYYYGSLYFDV

SEQ ID NO: 68 - protein, 11 aa, synthetic construct
RASENIYSYLA

SEQ ID NO: 69 - protein, 7 aa, synthetic construct
DAKTLAE

SEQ ID NO: 70 - protein, 9 aa, synthetic construct
QHHYGIPIT

SEQ ID NO: 71 - protein, 121 aa, synthetic construct
EVKLVESEGGLVQPGSSMKLSCTASGFTFSDFYMAWVRQVPEKGLEWVANINYDSTITYYLDSLKSRFIISRDNAENILYLQMSSLKSEDTATYYCARLLYYYGSLYFDVWGTGTTVTVSS

SEQ ID NO: 72 - protein, 107 aa, synthetic construct
DIQMTQSPASLSASVGETVTITCRASENIYSYLAWYQQKQGKSPQLLVYDAKTLAEGVPSRFSGSGSGTQFSLKINSLQPEDFGSYYCQHHYGIPITFGAGTNLELK

SEQ ID NO: 73 - protein, 5 aa, synthetic construct
NYWMH

SEQ ID NO: 74 - protein, 17 aa, synthetic construct
YINPSSGYTKYNQKFKD

SEQ ID NO: 75 - protein, 14 aa, synthetic construct
SLNYYDSGYWYFDV

SEQ ID NO: 76 - protein, 15 aa, synthetic construct
RASQSVSTSSYSYMH

SEQ ID NO: 77 - protein, 7 aa, synthetic construct
YASNLES

SEQ ID NO: 78 - protein, 9 aa, synthetic construct
QHSWEIPWT

SEQ ID NO: 79 - protein, 123 aa, synthetic construct
QVQLQQSGAELAKPGASVKLSCRTSGYTFTNYWMHWVKQRPGQGLEWIGYINPSSGYTKYNQKFKDKATLTADKSSSTAYMQLSSLTYEDSAVHYCARSLNYYDSGYWYFDVWGTGTAVTVSS

SEQ ID NO: 80 - protein, 111 aa, synthetic construct
DIVLTQSPASLAVSLGQRATISCRASQSVSTSSYSYMHWYQQKPGQPPKLLIKYASNLESRVPARFSGSGSGTDFTLNIHPVEEEDSATYYCQHSWEIPWTFGGGTKLEIK

SEQ ID NO: 81 - protein, 5 aa, synthetic construct
DYTMH

SEQ ID NO: 82 - protein, 17 aa, synthetic construct
GINPNYGGTSYNETFKD

SEQ ID NO: 83 - protein, 10 aa, synthetic construct
IPYGSYPMDY

SEQ ID NO: 84 - protein, 17 aa, synthetic construct
KSSQSLLYSSNQKIYLA

SEQ ID NO: 85 - protein, 7 aa, synthetic construct
WASTRES

SEQ ID NO: 86 - protein, 8 aa, synthetic construct
QQYYRYRT

SEQ ID NO: 87 - protein, 119 aa, synthetic construct
AVQLQQSGPELLKPGASVKISCKASGYTFTDYTMHWVKQSHGKSLEWIGGINPNYGGTSYNETFKDKATLTVDKSSNTAYMELRSLTSEDSAVYYCARIPYGSYPMDYWGQGTSVTVSS

SEQ ID NO: 88 - protein, 112 aa, synthetic construct
DIVMSQSPSSLTVSVGEKVTMSCKSSQSLLYSSNQKIYLAWYQQKPGQSPKLLISWASTRESGVPDRFTGSGSGTDFTLTISSVKAEDLADYYCQQYYRYRTFGGGTKLEIK

SEQ ID NO: 89 - protein, 5 aa, synthetic construct
DHTIH

SEQ ID NO: 90 - protein, 17 aa, synthetic construct
YIYPVYGYTQNNEKFKG

SEQ ID NO: 91 - protein, 11 aa, synthetic construct
SRDSNPYYFDY

SEQ ID NO: 92 - protein, 12 aa, synthetic construct
TVSSSISSSNLH

SEQ ID NO: 93 - protein, 7 aa, synthetic construct
GTSNLAS

SEQ ID NO: 94 - protein, 9 aa, synthetic construct
QQWSSYPFT

SEQ ID NO: 95 - protein, 120 aa, synthetic construct
QVQLQQSDAELVKPGASVKISCKASGSTFTDHTIHWVKQRPEQGLEWIGYIYPVYGYTQNNEKFKGKATLTADKSSSTAYMQLNSLTSEDSAVYFCARSRDSNPYYFDYWGQGTTLTVSS

SEQ ID NO: 96 - protein, 108 aa, synthetic construct
EIVLTQSPALMAASPGEKVTITCTVSSSISSSNLHWYQQKSGTSPKPWIYGTSNLASGVPVRFSGSGSGTSYSLTISSMEAEDAATYYCQQWSSYPFTFGSGTKLKMK

SEQ ID NO: 97 - protein, 5 aa, synthetic construct
DYNMH

SEQ ID NO: 98 - protein, 17 aa, synthetic construct
YIYRNNGYNGYNQKFKN

SEQ ID NO: 99 - protein, 9 aa, synthetic construct
NYWRGAMDY

SEQ ID NO: 100 - protein, 10 aa, synthetic construct
SASSSISYMH

SEQ ID NO: 101 - protein, 7 aa, synthetic construct
DTSKLAS

SEQ ID NO: 102 - protein, 9 aa, synthetic construct
HQRSSYPWT

SEQ ID NO: 103 - protein, 118 aa, synthetic construct
EVQLQQSGPELVKPGASVKISCKASGYTFTDYNMHWVKQSHGKSLEWIGYIYRNNGYNGYNQKFKNKATLTVDSSSSTAYMELRSLTSEDSAVYYCARNYWRGAMDYWGQGTSVTVSS

SEQ ID NO: 104 - protein, 106 aa, synthetic construct
QIVLTQSPAIMSASPGEKVTMTCSASSSISYMHWYQQKPGTSPKRWIYDTSKLASGVPARFSGSGSGTSYSLTISSMEAEDAGTYYCHQRSSYPWTFGGGTKLEIK

SEQ ID NO: 105 - protein, 5 aa, synthetic construct
SYTMH

SEQ ID NO: 106 - protein, 17 aa, synthetic construct
YIDPKSDYNYYNQKFKD

SEQ ID NO: 107 - protein, 9 aa, synthetic construct
GFFKGYFDV

SEQ ID NO: 108 - protein, 12 aa, synthetic construct
SVSSSISSSNLH

SEQ ID NO: 109 - protein, 7 aa, synthetic construct
GTSNLAS

SEQ ID NO: 110 - protein, 9 aa, synthetic construct
QQWTSYPFT

SEQ ID NO: 111 - protein, 118 aa, synthetic construct
QVQLQQSGAELARPGASVKMSCKASGYTFTSYTMHWVKQRPGQGLEWIGYIDPKSDYNYYNQKFKDKATLTADKSSSTAYMQLSGLTSEDSTVYYCARGFFKGYFDVWGAGTTVTVSS

SEQ ID NO: 112 - protein, 108 aa, synthetic construct
EIVLTQSPPLMAASPGEKVTITCSVSSSISSSNLHWYQQKSETSPKPWIYGTSNLASGVPIRFSGSGSGTSYSLTISSMEAEDAATYYCQQWTSYPFTFGAGTKLELK

SEQ ID NO: 113 - protein, 119 aa, synthetic construct
QVQLVQSGAEVKKPGASVKVSCKASGYTFTDHTIHWVRQAPGQGLEWMGYIYPRDGYTKYNEKFKDRVTMTTDTSTSTAYMELRSLRSDDTAVYYCARFYYGYWYFDVWGQGTTVTVSS

SEQ ID NO: 114 - protein, 119 aa, synthetic construct
QVQLVQSGAEVKKPGASVKVSCKASGYTFTDHTIHWVRQAPGQGLEWIGYIYPRDGYTKYNEKFKDRATMTTDTSTSTAYMELRSLRSDDTAVYYCARFYYGYWYFDVWGQGTTVTVSS

SEQ ID NO: 115 - protein, 119 aa, synthetic construct
QVQLVQSGAEVKKPGASVKVSCKASGYTFTDHTIHWMRQAPGQGLEWIGYIYPRDGYTKYNEKFKDRATMTTDTSTSTAYMELRSLRSDDTAVYYCARFYYGYWYFDVWGQGTTVTVSS

SEQ ID NO: 116 - protein, 119 aa, synthetic construct
QVQLVQSGAEVKKPGASVKVSCKASGYTFTDHTIHWMRQRPGQGLEWIGYIYPRDGYTKYNEKFKDRATLTADTSTSTAYMELRSLRSDDTAVYYCARFYYGYWYFDVWGQGTTVTVSS

SEQ ID NO: 117 - protein, 119 aa, synthetic construct
QVQLVQSGAEVKKPGASVKVSCKASGYTFTDHTIHWMRQRPGQGLEWIGYIYPRDGYTKYNEKFKDKATLTADKSTSTAYMELRSLRSDDTAVYYCARFYYGYWYFDVWGQGTTVTVSS

SEQ ID NO: 118 - protein, 119 aa, synthetic construct
QVQLVQSGAEVKKPGASVKVSCKVSGYTFTDHTIHWMKQRPGQGLEWIGYIYPRDGYTKYNEKFKDKATLTADKSTSTAYIELNSLRSDDTAVYFCARFYYGYWYFDVWGQGTTVTVSS

SEQ ID NO: 119 - protein, 119 aa, synthetic construct
QVQLVQSGAEVKKPGASVKVSCKASGYTFTDHTIHWVRQAPGQGLEWMGYIYPRDGYTKYNEKFKDRVTLTADKSTSTAYMELNSLTSEDTAVYFCARFYYGYWYFDVWGRGTLVTVSS

SEQ ID NO: 120 - protein, 98 aa, synthetic construct
QVQLVQSGAEVKKPGASVKVSCKASGYTFTSYGISWVRQAPGQGLEWMGWISAYNGNTNYAQKLQGRVTMTTDTSTSTAYMELRSLRSDDTAVYYCAR

SEQ ID NO: 121 - protein, 112 aa, synthetic construct
DIVMTQSPLSLPVTPGEPASISCRSSKSLLRSNGNTYLYWYLQKPGQSPQLLIYRMSNLASGVPDRFSGSGSGTDFTLKISRVEAEDVGVYYCMQHLEYPFTFGQGTKLEIK

SEQ ID NO: 122 - protein, 112 aa, synthetic construct
DIVMTQSPLSLPVTPGEPASISCRSSKSLLRSNGNTYLYWYLQKPGQSPQVLIYRMSNLASGVPDRFSGSGSGTDFTLKISRVEAEDVGVYYCMQHLEYPFTFGQGTKLEIK

SEQ ID NO: 123 - protein, 112 aa, synthetic construct
DIVMTQSPLSLPVTPGEPASISCRSSKSLLRSNGNTYLYWFLQKPGQSPQVLIYRMSNLASGVPDRFSGSGSGTDFTLKISRVEAEDVGVYYCMQHLEYPFTFGQGTKLEIK

SEQ ID NO: 124 - protein, 100 aa, synthetic construct
DIVMTQSPLSLPVTPGEPASISCRSSQSLLHSNGYNYLDWYLQKPGQSPQLLIYLGSNRASGVPDRFSGSGSGTDFTLKISRVEAEDVGVYYCMQALQTP

SEQ ID NO: 125 - protein, 121 aa, synthetic construct
QVQLVQSGAEVKKPGASVKVSCKASGYTFTDYDMHWVRQAPGQGLEWMGGFDPESAGTVYNLRFKDRVTMTTDTSTSTAYMELRSLRSDDTAVYYCARKGYYSVSSPFTYWGQGTLVTVSS

SEQ ID NO: 126 - protein, 121 aa, synthetic construct
QVQLVQSGAEVKKPGASVKVSCKASGYTFTDYDMHWVRQAPGQGLEWIGGFDPESAGTVYNLRFKDRVTMTTDTSTSTAYMELRSLRSDDTAVYYCARKGYYSVSSPFTYWGQGTLVTVSS

SEQ ID NO: 127 - protein, 121 aa, synthetic construct
QVQLVQSGAEVKKPGASVKVSCKASGYTFTDYDMHWVRQAPGQGLEWIGGFDPESAGTVYNLRFKDRATMTTDTSTSTAYMELRSLRSDDTAVYYCARKGYYSVSSPFTYWGQGTLVTVSS

SEQ ID NO: 128 - protein, 121 aa, synthetic construct
QVQLVQSGAEVKKPGASVKVSCKASGYTFTDYDMHWVKQAPGQGLEWIGGFDPESAGTVYNLRFKDRATLTTDTSTSTAYMELRSLRSDDTAVYYCARKGYYSVSSPFTYWGQGTLVTVSS

SEQ ID NO: 129 - protein, 121 aa, synthetic construct
QVQLVQSGAEVKKPGASVKVSCKASGYTFTDYDMHWVKQAPGQGLEWIGGFDPESAGTVYNLRFKDKATLTTDTSTSTAYMELRSLRSDDTAVYYCARKGYYSVSSPFTYWGQGTLVTVSS

SEQ ID NO: 130 - protein, 121 aa, synthetic construct
QVQLVQSGAEVKKPGASVKVSCKASGYTFTDYDMHWVKQAPGQGLEWIGGFDPESAGTVYNLRFKDKATLTTDKSTSTAYMELRSLRSDDTAVYYCARKGYYSVSSPFTYWGQGTLVTVSS

SEQ ID NO: 131 - protein, 121 aa, synthetic construct
QVQLVQSGAEVKKPGASVKVSCKASGYTFTDYDMHWVKQAPGQGLEWIGGFDPESAGTVYNLRFKDKATLTADKSTSTAYMELRSLRSEDTAVYYCARKGYYSVSSPFTYWGQGTLVTVSS

SEQ ID NO: 132 - protein, 121 aa, synthetic construct
QVQLVQSGAEVKKPGASVKVSCKASGYTFTDYDMHWVRQAPGKGLEWMGGFDPESAGTVYNLRFKDRVTLTADKSTSTAYMELRSLTSEDTAVYYCARKGYYSVSSPFTYWGQGTLVTVSS

SEQ ID NO: 133 - protein, 98 aa, synthetic construct; identical to SEQ ID NO: 120

SEQ ID NO: 134 - protein, 113 aa, synthetic construct
DIVMTQSPDSLAVSLGERATINCKSSQSLLYSSNQKNYLAWYQQKPGQPPKLLIYWASTRESGVPDRFSGSGSGTDFTLTISSLQAEDVAVYYCQQCYSYPRTFGGGTKVEIK

SEQ ID NO: 135 - protein, 113 aa, synthetic construct
DIVMTQSPDSLAVSLGERATINCKSSQSLLYSSNQKNYLAWYQQKPGQSPKLLIYWASTRESGVPDRFSGSGSGTDFTLTISSLQAEDVAVYYCQQCYSYPRTFGGGTKVEIK

SEQ ID NO: 136 - protein, 113 aa, synthetic construct
DIGMTQSPDSLAVSLGERATINCKSSQSLLYSSNQKNYLAWYQQKPGQSPKLLIYWASTRESGVPDRFSGSGSGTDFTLTISSLQAEDVAVYYCQQCYSYPRTFGGGTKVEIK

SEQ ID NO: 137 - protein, 113 aa, synthetic construct
DIGMSQSPDSLAVSLGERATINCKSSQSLLYSSNQKNYLAWYQQKPGQSPKLLIYWASTRESGVPDRFSGSGSGTDFTLTISSLQAEDVAVYYCQQCYSYPRTFGGGTKVEIK

SEQ ID NO: 138 - protein, 101 aa, synthetic construct
DIVMTQSPDSLAVSLGERATINCKSSQSVLYSSNNKNYLAWYQQKPGQPPKLLIYWASTRESGVPDRFSGSGSGTDFTLTISSLQAEDVAVYYCQQYYSTP

SEQ ID NO: 139 - protein, 119 aa, synthetic construct
EVQLVESGGGLVKPGGSLRLSCAASGFTFSSYAMSWVRQAPGKGLEWVSTINIGGSYTYYPDSVKGRFTISRDNAKNSLYLQMNSLRAEDTAVYYCARQEGRYWYFDVWGQGTTVTVSS

SEQ ID NO: 140 - protein, 119 aa, synthetic construct
EVQLVESGGGLVKPGGSLRLSCAASGFTFSSYAMSWVRQAPGKGLEWVATINIGGSYTYYPDSVKGRFTISRDNAKNSLYLQMNSLRAEDTAVYYCARQEGRYWYFDVWGQGTTVTVSS

SEQ ID NO: 141 - protein, 98 aa, synthetic construct
EVQLVESGGGLVKPGGSLRLSCAASGFTFSSYSMNWVRQAPGKGLEWVSSISSSSSYIYYADSVKGRFTISRDNAKNSLYLQMNSLRAEDTAVYYCAR

SEQ ID NO: 142 - protein, 108 aa, synthetic construct
DIQLTQSPSFLSASVGDRVTITCTASSSVSSSYLHWYQQKPGKAPKLLIYSTSNLASGVPSRFSGSGSGTEFTLTISSLQPEDFATYYCHQFHRSPYTFGGGTKVEIK

SEQ ID NO: 143 - protein, 108 aa, synthetic construct
DIQLTQSPSFLSASVGDRVTITCTASSSVSSSYLHWYQQKPGKAPKLWIYSTSNLASGVPSRFSGSGSGTEYTLTISSLQPEDFATYYCHQFHRSPYTFGGGTKVEIK

SEQ ID NO: 144 - protein, 108 aa, synthetic construct
DIVLTQSPSFLSASVGDRVTITCTASSSVSSSYLHWYQQKPGKSPKLWIYSTSNLASGVPSRFSGSGSGTEYSLTISSLQPEDFATYYCHQFHRSPYTFGGGTKVEIK

SEQ ID NO: 145 - protein, 108 aa, synthetic construct
QIVLTQSPSFLSASVGDRVTITCTASSSVSSSYLHWYQQKPGKSPKLWIYSTSNLASGVPSRFSGSGSGTSYSLTISSLQPEDFATYYCHQFHRSPYTFGGGTKVEIK

SEQ ID NO: 146 - protein, 96 aa, synthetic construct
DIQLTQSPSFLSASVGDRVTITCRASSQGISSYLAWYQQKPGKAPKLLIYAASTLQSGVPSRFSGSGSGTEFTLTISSLQPEDFATYYCQQLNSYP

SEQ ID NO: 147 - protein, 108 aa, synthetic construct
EIVLTQSPGTLSLSPGERATLSCTASSSVSSSYLHWYQQKPGQAPRLLIYSTSNLASGIPDRFSGSGSGTDFTLTISRLEPEDFAVYYCHQFHRSPYTFGGGTKVEIK

SEQ ID NO: 148 - protein, 96 aa, synthetic construct
EIVLTQSPGTLSLSPGERATLSCRASQSVSSSYLAWYQQKPGQAPRLLIYGASSRATGIPDRFSGSGSGTDFTLTISRLEPEDFAVYYCQQYGSYT

SEQ ID NO: 149 - protein, 115 aa, synthetic construct
QVQLVQSGAEVKKPGASVKVSCKASGYTFTTYWMHWVRQAPGQRLEWMGEIDPSDSYANYNQKFKGRVTITRDTSASTAYMELSSLRSEDTAVYYCARYYGYGDWGQGTTVTVSS

SEQ ID NO: 150 - protein, 115 aa, synthetic construct
QVQLVQSGAEVKKPGASVKVSCKASGYTFTTYWMHWVRQAPGQRLEWIGEIDPSDSYANYNQKFKGRATITRDTSASTAYMELSSLRSEDTAVYYCALYYGYGDWGQGTTVTVSS

SEQ ID NO: 151 - protein, 115 aa, synthetic construct
QVQLVQSGAEVKKPGASVKVSCKASGYTFTTYWMHWVRQAPGQRLEWIGEIDPSDSYANYNQKFKGKATLTVDTSASTAYMELSSLRSEDTAVYYCALYYGYGDWGQGTTVTVSS

SEQ ID NO: 152 - protein, 115 aa, synthetic construct
QVQLVQSGAEVKKPGASVKVSCKASGYTFTTYWMHWVKQAPGQRLEWIGEIDPSDSYANYNQKFKGKATLTVDKSASTAYMELSSLRSEDTAVYYCALYYGYGDWGQGTTVTVSS

SEQ ID NO: 153 - protein, 98 aa, synthetic construct
QVQLVQSGAEVKKPGASVKVSCKASGYTFTSYAMHWVRQAPGQRLEWMGWINAGNGNTKYSQKFQGRVTITRDTSASTAYMELSSLRSEDTAVYYCAR

SEQ ID NO: 154 - protein, 115 aa, synthetic construct
QVQLVQSGAEVKKPGASVKVSCKASGYTFTTYWMHWVRQAPGQGLEWMGEIDPSDSYANYNQKFKGRVTLTRDTSTSTAYMELSSLTSEDTAVYYCARYYGYGDWGQGTTVTVSS

SEQ ID NO: 155 - protein, 99 aa, synthetic construct
QVQLVQSGAEVKKPGASVKVSCKASGYTFTSYYMHWVRQAPGQGLEWMGIINPSGGSTSYAQKFQGRVTMTRDTSTSTVYMELSSLRTSEDTAVYYCAR

SEQ ID NO: 156 - protein, 108 aa, synthetic construct
EIVLTQSPDFQSVTPKEKVTITCSVSSSISSIHLHWYQQKPDQSPKLLIKRTSNLASGVPSRFSGSGSGTDFTLTINSLEAEDAATYYCQQGSNLPLTFGQGTRLEIK

SEQ ID NO: 157 - protein, 108 aa, synthetic construct
EIVLTQSPDFQSVTPKEKVTITCSVSSSISSIHLHWYQQKPDQSPKLLIYRTSNLASGVPSRFSGSGSGTDFTLTINSLEAEDAATYYCQQGSNLPLTFGQGTRLEIK

SEQ ID NO: 158 - protein, 108 aa, synthetic construct
EIVLTQSPDFQSVTPKEKVTITCSVSSSISSIHLHWYQQKPDQSPKLLIYRTSNLASGVPSRFSGSGSGTDYTLTINSLEAEDAATYYCQQGSNLPLTFGQGTRLEIK

SEQ ID NO: 159 - protein, 95 aa, synthetic construct
EIVLTQSPDFQSVTPKEKVTITCRASQSIGSSLHWYQQKPDQSPKLLIKYASQSFSGVPSRFSGSGSGTDFTLTINSLEAEDAATYYCHQSSSLP

SEQ ID NO: 160 - protein, 108 aa, synthetic construct
EIVLTQSPGTLSLSPGERATLSCSVSSSISSIHLHWYQQKPGQAPRLLIYRTSNLASGIPDRFSGSGSGTDFTLTISRLEPEDFAVYYCQQGSNLPLTFGQGTRLEIK

SEQ ID NO: 161 - protein, 96 aa, synthetic construct
EIVLTQSPGTLSLSPGERATLSCRASQSVSSSYLAWYQQKPGQAPRLLIYGASSRATGIPDRFSGSGSGTDFTLTISRLEPEDFAVYYCQQYGSSP

SEQ ID NO: 162 - protein, 120 aa, synthetic construct
QVQLVQSGAEVKKPGSSVKVSCKASGSTFTDHTIHWVRQAPGQGLEWMGYIYPVYGYTQNNEKFKGRVTITADKSTSTAYMELSSLRSEDTAVYYCARSRDSNPYYFDYWGQGTTVTVSS

SEQ ID NO: 163 - protein, 120 aa, synthetic construct
QVQLVQSGAEVKKPGSSVKVSCKASGSTFTDHTIHWVRQAPGQGLEWIGYIYPVYGYTQNNEKFKGRATITADKSTSTAYMELSSLRSEDTAVYYCARSRDSNPYYFDYWGQGTTVTVSS

SEQ ID NO: 164 - protein, 120 aa, synthetic construct
QVQLVQSGAEVKKPGSSVKVSCKASGSTFTDHTIHWVRQAPGQGLEWIGYIYPVYGYTQNNEKFKGRATITADKSTSTAYMELNSLRSEDTAVYYCARSRDSNPYYFDYWGQGTTVTVSS

SEQ ID NO: 165 - protein, 120 aa, synthetic construct
QVQLVQSGAEVKKPGSSVKVSCKASGSTFTDHTIHWVKQAPGQGLEWIGYIYPVYGYTQNNEKFKGKATLTADKSTSTAYMELNSLRSEDTAVYFCARSRDSNPYYFDYWGQGTTVTVSS

SEQ ID NO: 166 - protein, 98 aa, synthetic construct
QVQLVQSGAEVKKPGSSVKVSCKASGGTFSSYTISWVRQAPGQGLEWMGRIIPILGIANYAQKFQGRVTITADKSTSTAYMELSSLRSEDTAVYYCAR

SEQ ID NO: 167 - protein, 108 aa, synthetic construct
EIVLTQSPDFQSVTPKEKVTITCTVSSSISSSNLHWYQQKPDQSPKLLIYGTSNLASGVPSRFSGSGSGTDFTLTINSLEAEDAATYYCQQWSSYPFTFGQGTKLEIK

SEQ ID NO: 168 - protein, 108 aa, synthetic construct
EIVLTQSPDFQSVTPKEKVTITCTVSSSISSSNLHWYQQKPDQSPKLWIYGTSNLASGVPSRFSGSGSGTDYTLTINSLEAEDAATYYCQQWSSYPFTFGQGTKLEIK

SEQ ID NO: 169 - protein, 108 aa, synthetic construct
EIVLTQSPDFQSVTPKEKVTITCTVSSSISSSNLHWYQQKPDQSPKPWIYGTSNLASGVPSRFSGSGSGTDYSLTINSLEAEDAATYYCQQWSSYPFTFGQGTKLEIK

SEQ ID NO: 170 - protein, 95 aa, synthetic construct; identical to SEQ ID NO: 159

SEQ ID NO: 171 - protein, 108 aa, synthetic construct
EIVLTQSPATLSLSPGERATLSCTVSSSISSSNLHWYQQKPGLAPRLLIYGTSNLASGIPDRFSGSGSGTDFTLTISRLEPEDFAVYYCQQWSSYPFTFGQGTKLEIK

SEQ ID NO: 172 - protein, 96 aa, synthetic construct
EIVLTQSPATLSLSPGERATLSCGASQSVSSSYLAWYQQKPGLAPRLLIYDASSRATGIPDRFSGSGSGTDFTLTISRLEPEDFAVYYCQQYGSSP

SEQ ID NO: 173 - protein, 118 aa, synthetic construct
QVQLVQSGAEVKKPGASVKVSCKASGYTFTDYNMHWVRQAPGQRLEWMGYIYRNNGYNGYNQKFKNRVTITRDTSASTAYMELSSLRSEDTAVYYCARNYWRGAMDYWGQGTTVTVSS

SEQ ID NO: 174 - protein, 118 aa, synthetic construct
QVQLVQSGAEVKKPGASVKVSCKASGYTFTDYNMHWVRQAPGQRLEWIGYIYRNNGYNGYNQKFKNRATITRDTSASTAYMELSSLRSEDTAVYYCARNYWRGAMDYWGQGTTVTVSS

SEQ ID NO: 175 - protein, 118 aa, synthetic construct
QVQLVQSGAEVKKPGASVKVSCKASGYTFTDYNMHWVKQAPGQRLEWIGYIYRNNGYNGYNQKFKNRATLTRDTSASTAYMELSSLRSEDTAVYYCARNYWRGAMDYWGQGTTVTVSS

SEQ ID NO: 176 - protein, 118 aa, synthetic construct
QVQLVQSGAEVKKPGASVKVSCKASGYTFTDYNMHWVKQAPGQRLEWIGYIYRNNGYNGYNQKFKNKATLTVDTSASTAYMELSSLRSEDTAVYYCARNYWRGAMDYWGQGTTVTVSS

SEQ ID NO: 177 - protein, 98 aa, synthetic construct; identical to SEQ ID NO: 153

SEQ ID NO: 178 - protein, 106 aa, synthetic construct
EIVLTQSPATLSLSPGERATLSCSASSSISYMHWYQQKPGKAPKLLIYDTSKLASGVPSRFSGSGSGTDFTLTISSLQPEDFATYYCHQRSSYPWTFGGGTKVEIK

SEQ ID NO: 179 - protein, 106 aa, synthetic construct
EIVLTQSPATLSLSPGERATLSCSASSSISYMHWYQQKPGKAPKRLIYDTSKLASGVPSRFSGSGSGTDFTLTISSLQPEDFATYYCHQRSSYPWTFGGGTKVEIK

SEQ ID NO: 180 - protein, 106 aa, synthetic construct
EIVLTQSPATLSLSPGERATLSCSASSSISYMHWYQQKPGKAPKRWIYDTSKLASGVPSRFSGSGSGTDFTLTISSLQPEDFATYYCHQRSSYPWTFGGGTKVEIK

SEQ ID NO: 181 - protein, 106 aa, synthetic construct
EIVLTQSPATLSLSPGERATLSCSASSSISYMHWYQQKPGKAPKRWIYDTSKLASGVPSRFSGSGSGTDYTLTISSLQPEDFATYYCHQRSSYPWTFGGGTKVEIK

SEQ ID NO: 182 - protein, 95 aa, synthetic construct
AIQLTQSPSSLSASVGDRVTITCRASQGISSALAWYQQKPGKAPKLLIYDASSLESGVPSRFSGSGSGTDFTLTISSLQPEDFATYYCQQFNSYP

SEQ ID NO: 183 - protein, 106 aa, synthetic construct
EIVLTQSPATLSLSPGERATLSCSASSSISYMHWYQQKPGQAPRLLIYDTSKLASGIPARFSGSGSGTDFTLTISSLEPEDFAVYYCHQRSSYPWTFGGGTKVEIK

SEQ ID NO: 184 - protein, 106 aa, synthetic construct
EIVLTQSPATLSLSPGERATLSCSASSSISYMHWYQQKPGQAPRLWIYDTSKLASGVPARFSGSGSGTDFTLTISSLEPEDFAVYYCHQRSSYPWTFGGGTKVEIK

SEQ ID NO: 185 - protein, 95 aa, synthetic construct
EIVLTQSPATLSLSPGERATLSCRASQSVSSYLAWYQQKPGQAPRLLIYDASNRATGIPARFSGSGSGTDFTLTISSLEPEDFAVYYCQQRSNWP

SEQ ID NO: 186 - protein, 118 aa, synthetic construct
QVQLVQSGAEVKKPGASVKVSCKASGYTFTSYTMHWVRQAPGQGLEWMGYIDPKSDYNYYNQKFKDRVTMTRDTSISTAYMELSRLRSDDTAVYYCARGFFKGYFDVWGQGTTVTVSS

SEQ ID NO: 187 - protein, 118 aa, synthetic construct
QVQLVQSGAEVKKPGASVKVSCKASGYTFTSYTMHWVRQAPGQGLEWIGYIDPKSDYNYYNQKFKDRATLTRDTSISTAYMELSRLRSDDTAVYYCARGFFKGYFDVWGQGTTVTVSS

SEQ ID NO: 188 - protein, 118 aa, synthetic construct
QVQLVQSGAEVKKPGASVKVSCKASGYTFTSYTMHWVKQAPGQGLEWIGYIDPKSDYNYYNQKFKDKATLTADTSISTAYMELSRLRSDDTAVYYCARGFFKGYFDVWGQGTTVTVSS

SEQ ID NO: 189 - protein, 118 aa, synthetic construct
QVQLVQSGAEVKKPGASVKVSCKASGYTFTSYTMHWVKQAPGQGLEWIGYIDPKSDYNYYNQKFKDKATLTADKSISTAYMELSRLRSDDTAVYYCARGFFKGYFDVWGQGTTVTVSS

SEQ ID NO: 190 - protein, 98 aa, synthetic construct
QVQLVQSGAEVKKPGASVKVSCKASGYTFTGYYMHWVRQAPGQGLEWMGWINPNSGGTNYAQKFQGRVTMTRDTSISTAYMELSRLRSDDTAVYYCAR

SEQ ID NO: 191 - protein, 118 aa, synthetic construct
QVQLVQSGAEVKKPGASVKVSCKASGYTFTSYTMHWVRQAPGQGLEWMGYIDPKSDYNYYNQKFKDRVTLTADKSTSTAYMELSGLTSEDTAVYYCARGFFKGYFDVWGQGTTVTVSS

SEQ ID NO: 192 - protein, 98 aa, synthetic construct
QVQLVQSGAEVKKPGASVKVSCKASGYTFTSYYMHWVRQAPGQGLEWMGIINPSGGSTSYAQKFQGRVTMTRDTSTSTVYMELSSLRSEDTAVYYCAR

SEQ ID NO: 193 - protein, 108 aa, synthetic construct
EIVLTQSPGTLSLSPGERATLSCSVSSSISSSNLHWYQQKPGQAPRLLIYGTSNLASGIPDRFSGSGSGTDFTLTISRLEPEDFAVYYCQQWTSYPFTFGQGTKLEIK

SEQ ID NO: 194 - protein, 108 aa, synthetic construct
EIVLTQSPGTLSLSPGERATLSCSVSSSISSSNLHWYQQKPGQAPRLWIYGTSNLASGVPDRFSGSGSGTDFTLTISRLEPEDFAVYYCQQWTSYPFTFGQGTKLEIK

SEQ ID NO: 195 - protein, 108 aa, synthetic construct
EIVLTQSPGTLSLSPGERATLSCSVSSSISSSNLHWYQQKPGQAPRPWIYGTSNLASGVPDRFSGSGSGTDYTLTISRLEPEDFAVYYCQQWTSYPFTFGQGTKLEIK

SEQ ID NO: 196 - protein, 108 aa, synthetic construct
EIVLTQSPGTLSLSPGERATLSCSVSSSISSSNLHWYQQKPGQSPRPWIYGTSNLASGVPDRFSGSGSGTSYTLTISRLEPEDFAVYYCQQWTSYPFTFGQGTKLEIK

SEQ ID NO: 197 - protein, 96 aa, synthetic construct; identical to SEQ ID NO: 148

SEQ ID NO: 198 - protein, 108 aa, synthetic construct
EIVLTQSPDFQSVTPKEKVTITCSVSSSISSSNLHWYQQKPDQSPKLLIKGTSNLASGVPSRFSGSGSGTDFTLTINSLEAEDAATYYCQQWTSYPFTFGQGTKLEIK

SEQ ID NO: 199 - protein, 108 aa, synthetic construct
EIVLTQSPDFQSVTPKEKVTITCSVSSSISSSNLHWYQQKPDQSPKPWIYGTSNLASGVPSRFSGSGSGTDYTLTINSLEAEDAATYYCQQWTSYPFTFGQGTKLEIK

SEQ ID NO: 200 - protein, 95 aa, synthetic construct; identical to SEQ ID NO: 159

SEQ ID NO: 201 - protein, 112 aa, synthetic construct
DIVMTQSPLSLPVTPGEPASISCRSSKSLLRSNGNTYLYWFLQKPGQSPQVLIYRMSNLASGVPDRFSGSGSGTAFTLKISRVEAEDVGVYYCMQHLEYPFTFGQGTKLEIK

SEQ ID NO: 202 - protein, 112 aa, synthetic construct
DIVMTQSPLSLPVTPGEPASISCRSSKSLLRSNGNTYLYWFLQKPGQSPQVLIYRMSNLASGVPDRFSGSGSGTAFTLKISRVEAEDVGVYYCMQHLEYPFTFGAGTKLEIK

SEQ ID NO: 203 - protein, 113 aa, synthetic construct
DIVMTQSPDSLAVSLGERATINCKSSQSLLYSSNQKNYLAWYQQKPGQPPKLLIYWASTRESGVPDRFSGSGSGTDFTLTISSLQAEDVAVYYCQQHYSYPRTFGGGTKVEIK

SEQ ID NO: 204 - protein, 113 aa, synthetic construct
DIVMTQSPDSLAVSLGERATINCKSSQSLLYSSNQKNYLAWYQQKPGQPPKLLIYWASTRESGVPDRFSGSGSGTDFTLTISSLQAEDVAVYYCQQLYSYPRTFGGGTKVEIK

SEQ ID NO: 205 - protein, 113 aa, synthetic construct
DIVMTQSPDSLAVSLGERATINCKSSQSLLYSSNQKNYLAWYQQKPGQPPKLLIYWASTRESGVPDRFSGSGSGTDFTLTISSLQAEDVAVYYCQQYYSYPRTFGGGTKVEIK

SEQ ID NO: 206 - protein, 113 aa, synthetic construct
DIVMTQSPDSLAVSLGERATINCKSSQSLLYSSNQKNYLAWYQQKPGQPPKLLIYWASTRESGVPDRFSGSGSGTDFTLTISSLQAEDVAVYYCQQSYSYPRTFGGGTKVEIK

SEQ ID NO: 207 - protein, 113 aa, synthetic construct
DIVMTQSPDSLAVSLGERATINCKSSQSLLYSSNQKNYLAWYQQKPGQPPKLLIYWASTRESGVPDRFSGSGSGTDFTLTISSLQAEDVAVYYCQQTYSYPRTFGGGTKVEIK

SEQ ID NO: 208 - protein, 112 aa, synthetic construct
DIVMTQSPLSLPVTPGEPASISCRSSKSLLRSNGNTYLYWFLQKPGQSPQVLIYRMSNLASGVPDRFSGSGSGTDFTLKISRVEAEDVGVYYCHQHLEYPFTFGQGTKLEIK

SEQ ID NO: 209 - protein, 112 aa, synthetic construct
DIVMTQSPLSLPVTPGEPASISCRSSKSLLRSNGNTYLYWFLQKPGQSPQVLIYRMSNLASGVPDRFSGSGSGTDFTLKISRVEAEDVGVYYCKQHLEYPFTFGQGTKLEIK

SEQ ID NO: 210 - protein, 112 aa, synthetic construct
DIVMTQSPLSLPVTPGEPASISCRSSKSLLRSNGNTYLYWFLQKPGQSPQVLIYRMSNLASGVPDRFSGSGSGTDFTLKISRVEAEDVGVYYCSQHLEYPFTFGQGTKLEIK

SEQ ID NO: 211 - protein, 112 aa, synthetic construct
DIVMTQSPLSLPVTPGEPASISCRSSKSLLRSNGNTYLYWFLQKPGQSPQVLIYRMSNLASGVPDRFSGSGSGTDFTLKISRVEAEDVGVYYCTQHLEYPFTFGQGTKLEIK

SEQ ID NO: 212 - protein, 112 aa, synthetic construct
DIVMTQSPLSLPVTPGEPASISCRSSKSLLRSNGNTYLYWFLQKPGQSPQVLIYRMSNLASGVPDRFSGSGSGTDFTLKISRVEAEDVGVYYCNQHLEYPFTFGQGTKLEIK

SEQ ID NO: 213 - protein, 112 aa, synthetic construct
DIVMTQSPLSLPVTPGEPASISCRSSKSLLRSNGNTYLYWFLQKPGQSPQVLIYRMSNLASGVPDRFSGSGSGTDFTLKISRVEAEDVGVYYCQQHLEYPFTFGQGTKLEIK

SEQ ID NO: 214 - protein, 112 aa, synthetic construct
DIVMTQSPLSLPVTPGEPASISCRSSKSLLRSNGNTYLYWFLQKPGQSPQVLIYRMSNLASGVPDRFSGSGSGTDFTLKISRVEAEDVGVYYCGQHLEYPFTFGQGTKLEIK

SEQ ID NO: 215 - protein, 112 aa, synthetic construct
DIVMTQSPLSLPVTPGEPASISCRSSKSLLRSNGNTYLYWFLQKPGQSPQVLIYRMSNLASGVPDRFSGSGSGTDFTLKISRVEAEDVGVYYCIQHLEYPFTFGQGTKLEIK

SEQ ID NO: 216 - protein, 112 aa, synthetic construct
DIVMTQSPLSLPVTPGEPASISCRSSKSLLRSNGNTYLYWFLQKPGQSPQVLIYRMSNLASGVPDRFSGSGSGTDFTLKISRVEAEDVGVYYCLQHLEYPFTFGQGTKLEIK

SEQ ID NO: 217 - protein, 9 aa, synthetic construct
QQHYSYPRT

SEQ ID NO: 218 - protein, 9 aa, synthetic construct
QQLYSYPRT

SEQ ID NO: 219 - protein, 9 aa, synthetic construct
QQYYSYPRT

SEQ ID NO: 220 - protein, 9 aa, synthetic construct
QQSYSYPRT

SEQ ID NO: 221 - protein, 9 aa, synthetic construct
QQTYSYPRT

SEQ ID NO: 222 - protein, 9 aa, synthetic construct
HQHLEYPFT

SEQ ID NO: 223 - protein, 9 aa, synthetic construct
KQHLEYPFT

SEQ ID NO: 224 - protein, 9 aa, synthetic construct
SQHLEYPFT

SEQ ID NO: 225 - protein, 9 aa, synthetic construct
TQHLEYPFT

SEQ ID NO: 226 - protein, 9 aa, synthetic construct
NQHLEYPFT

SEQ ID NO: 227 - protein, 9 aa, synthetic construct
QQHLEYPFT

SEQ ID NO: 228 - protein, 9 aa, synthetic construct
GQHLEYPFT

SEQ ID NO: 229 - protein, 9 aa, synthetic construct
IQHLEYPFT

SEQ ID NO: 230 - protein, 9 aa, synthetic construct
LQHLEYPFT

SEQ ID NO: 231 - protein, 832 aa, synthetic construct
MILQAHLHSLCLLMLYLATGYGQEGKFSGPLKPMTFSIYEGQEPSQIIFQFKANPPAVTFELTGETDNIFVIEREGLLYYNRALDRETRSTHNLQVAALDANGIIVEGPVPITIKVKDINDNRPTFLQSKYEGSVRQNSRPGKPFLYVNATDLDDPATPNGQLYYQIVIQLPMINNVMYFQINNKTGAISLTREGSQELNPAKNPSYNLVISVKDMGGQSENSFSDTTSVDIIVTENIWKAPKPVEMVENSTDPHPIKITQVRWNDPGAQYSLVDKEKLPRFPFSIDQEGDIYVTQPLDREEKDAYVFYAVAKDEYGKPLSYPLEIHVKVKDINDNPPTCPSPVTVFEVQENERLGNSIGTLTAHDRDEENTANSFLNYRIVEQTPKLPMDGLFLIQTYAGMLQLAKQSLKKQDTPQYNLTIEVSDKDFKTLCFVQINVIDINDQIPIFEKSDYGNLTLAEDTNIGSTILTIQATDADEPFTGSSKILYHIIKGDSEGRLGVDTDPHTNTGYVIIKKPLDFETAAVSNIVFKAENPEPLVFGVKYNASSFAKFTLIVTDVNEAPQFSQHVFQAKVSEDVAIGTKVGNVTAKDPEGLDISYSLRGDTRGWLKIDHVTGEIFSVAPLDREAGSPYRVQVVATEVGGSSLSSVSEFHLILMDVNDNPPRLAKDYTGLFFCHPLSAPGSLIFEATDDDQHLFRGPHFTFSLGSGSLQNDWEVSKINGTHARLSTRHTEFEEREYVVLIRINDGGRPPLEGIVSLPVTFCSCVEGSCFRPAGHQTGIPTVGMAVGILLTTLLVIGIILAVVFIRIKKDKGKDNVESAQASEVKPLRS

SEQ ID NO: 232 - protein, 108 aa, synthetic construct
EIVLTQSPGTLSLSPGERATLSCSVSSSISKIHLHWYQQKPGQAPRLLIYRTSNLASGIPDRFSGSGSGTDFTLTISRLEPEDFAVYYCQQGSNLPLTFGQGTRLEIK

SEQ ID NO: 233 - protein, 108 aa, synthetic construct
EIVLTQSPGTLSLSPGERATLSCSVSSSISRIHLHWYQQKPGQAPRLLIYRTSNLASGIPDRFSGSGSGTDFTLTISRLEPEDFAVYYCQQGSNLPLTFGQGTRLEIK

SEQ ID NO: 234 - protein, 108 aa, synthetic construct
EIVLTQSPGTLSLSPGERATLSCSVSASISRIHLHWYQQKPGQAPRLLIYRTSNLASGIPDRFSGSGSGTDFTLTISRLEPEDFAVYYCQQGSNLPLTFGQGTRLEIK

SEQ ID NO: 235 - protein, 108 aa, synthetic construct
EIVLTQSPGTLSLSPGERATLSCSVSSSISSIHLHWYQQKPGQAPRLLIYRTRNLASGIPDRFSGSGSGTDFTLTISRLEPEDFAVYYCQQGSNLPLTFGQGTRLEIK

SEQ ID NO: 236 - protein, 108 aa, synthetic construct
EIVLTQSPGTLSLSPGERATLSCSVSSSISSIHLHWYQQKPGQAPRLLIYRTRNRASGIPDRFSGSGSGTDFTLTISRLEPEDFAVYYCQQGSNLPLTFGQGTRLEIK

SEQ ID NO: 237 - protein, 108 aa, synthetic construct
EIVLTQSPGTLSLSPGERATLSCSVSSSISSIHLHWYQQKPGQAPRLLIYRTKNLASGIPDRFSGSGSGTDFTLTISRLEPEDFAVYYCQQGSNLPLTFGQGTRLEIK

SEQ ID NO: 238 - protein, 108 aa, synthetic construct
EIVLTQSPGTLSLSPGERATLSCSVSASISRIHLHWYQQKPGQAPRLLIYRTRNRASGIPDRFSGSGSGTDFTLTISRLEPEDFAVYYCQQGSNLPLTFGQGTRLEIK

SEQ ID NO: 239 - protein, 12 aa, synthetic construct
SVSSSISKIHLH

SEQ ID NO: 240 - protein, 12 aa, synthetic construct
SVSSSISRIHLH

SEQ ID NO: 241 - protein, 12 aa, synthetic construct
SVSASISRIHLH

SEQ ID NO: 242 - protein, 7 aa, synthetic construct
RTRNLAS

SEQ ID NO: 243 - protein, 7 aa, synthetic construct
RTRNRAS

SEQ ID NO: 244 - protein, 7 aa, synthetic construct
RTKNLAS

SEQ ID NO: 245 - protein, 17 aa, synthetic construct
YIYPREGYTKYNEKFKD

SEQ ID NO: 246 - protein, 16 aa, synthetic construct
RSSKSLLRSNANTYLY

SEQ ID NO: 247 - protein, 16 aa, synthetic construct
RSSKSLLRSNAQTYLY

SEQ ID NO: 248 - protein, 119 aa, synthetic construct
QVQLVQSGAEVKKPGASVKVSCKASGYTFTDHTIHWMRQRPGQGLEWIGYIYPREGYTKYNEKFKDRATLTADTSTSTAYMELRSLRSDDTAVYYCARFYYGYWYFDVWGQGTTVTVSS

SEQ ID NO: 249 - protein, 112 aa, synthetic construct
DIVMTQSPLSLPVTPGEPASISCRSSKSLLRSNANTYLYWFLQKPGQSPQVLIYRMSNLASGVPDRFSGSGSGTDFTLKISRVEAEDVGVYYCMQHLEYPFTFGQGTKLEIK

SEQ ID NO: 250 - protein, 112 aa, synthetic construct
DIVMTQSPLSLPVTPGEPASISCRSSKSLLRSNAQTYLYWFLQKPGQSPQVLIYRMSNLASGVPDRFSGSGSGTDFTLKISRVEAEDVGVYYCMQHLEYPFTFGQGTKLEIK